European Patent Specification EP 3 928 095 B1, published June 11, 2025. Title: Use of BMMF Rep Protein as Biomarker for Breast Cancer. Applicant: Deutsches Krebsforschungszentrum. The sequence listing filed with the application follows.

SEQUENCE LISTING (15 sequences)

SEQ ID NO: 1 - protein, 324 aa, artificial sequence
  MSBI1 Rep protein
MSDLIVKDNALMNASYNLALVEQRLILLAIIEARETGKGINANDPLTVHASSYINQFNVERHTAYQALKDACKDLFARQFSYQEKRERGRINITSRWVSQIGYMDDTATVEIIFAPAVVPLITRLEEQFTQYDIEQISGLSSAYAVRMYELLICWRSTGKTPIIELDEFRKRIGVLDTEYTRTDNLKMRVIELALKQINEHTDITASYEQHKKGRVITGFSFKFKHKKQNSDKTPKNSDSSPRIVKHSQIPTNIVKQPENAKMSDLEHRASRVTGEIMRNRLSDRFKQGDESAIDMMKRIQSEIITDAIADQWESKLEEFGVVF

SEQ ID NO: 2 - protein, 18 aa, artificial sequence
  Rep peptide
EARETGKGINANDPLTVH

SEQ ID NO: 3 - protein, 20 aa, artificial sequence
  Rep peptide
KQINEHTDITASYEHKKGRT

SEQ ID NO: 4 - protein, 8 aa, artificial sequence
  His tag
GAHHHHHH

SEQ ID NO: 5 - protein, 11 aa, artificial sequence
  T7 tag
MASMTGGQQMG

SEQ ID NO: 6 - protein, 8 aa, artificial sequence
  FLAG tag
DYKDDDDK

SEQ ID NO: 7 - protein, 8 aa, artificial sequence
  Trep II tag
WSHPQFEK

SEQ ID NO: 8 - protein, 319 aa, artificial sequence
  MSBI2.176
MSKLVVKDNALMNASYNLDLVEQRLILLAIIEARESGKGINANDPLTVHAESYINQFGVHRVTAYQALKDACDNLFARQFSYQSKSEKGNIQNHRSRWVSEIIYIDTEATVKIIFAPAIVPLITRLEEQFTKYDIEQISDLSSAYAIRLYELLICWRSTGKTPIIGLGEFRNRVGVLDSEYHRIAHLKERVIEHSIKQINEHTDITATYEQHKKGRTITGFSFKFKQKKPKQAEIATETPKTATNDPDTTKPLTEPQIAKYSMILCKLGSISDLSNFPDYPAFANWIGNILRNPEKADEQIAKRIFTALKTETDYSKKN

SEQ ID NO: 9 - protein, 7 aa, artificial sequence
  MSBI1 epitope
NRLSDRF

SEQ ID NO: 10 - protein, 326 aa, artificial
  CMI1.252
MSDLIVKDNALMNASYNLALVEQRLILLAILEARETGKGINANDPLTVHASSYINQFNVERHTAYQALKDACKDLFARQFSYQEKRERGRINITSRWVSQIGYMDDTATVEIIFAPAVVPLITRLEEQFTQYDIEQISELSSAYAVRLYELLICWRSTGKTPIIDLTEFRKRLGVLDTEYTRTDNLKMRVIELGLKQINEHTDITASYEQHKKGRTITGFSFKFKQKKKTGAEMPKNSDSSPHIEKPSQIPANIAKQPENAKKDDLGHRASKITGLIMSNGLADRFKRGDESVIDMMKRIKEEITTDTTADQWENKLEEFGVIFQS

SEQ ID NO: 11 - protein, 324 aa, artificial
  CMI2.214
MSDLIVKDNALMNASYNLDLVEQRLILLAILEARETGKGINANDPLTVHAESYINQFGVARQTAYQALKDACKDLFARQFSYQEKRERGRANITSRWVSQIAYIDETATVEVIFAPAVVPLITRLEEQFTQYDIEQISGLSSAYAVRLYELLICWRSTGKTPVIELAEFRKRLGVLNDEYTRSDNFKKWIIENPIKQINEHTDITASYEQHKKGRTITGFSFKFKQKKKTEPETPKNSDSSQRIEKPSQIPANIVKQPENANLSDLQHRASKITGLIMSNRLSDRFKQGDESIMQMMARIQSEITTDSIADQWQSKLEEFGVVF

SEQ ID NO: 12 - protein, 324 aa, artificial
  CMI3.168
MSDLIVKDNALMNASYNLALVEQRLILLAILEARETGKGINANDPLTVHASSYINQFNVERHTAYQALKDACKDLFARQFSYQEKRERGRANITSRWVSQIAYIDETATVEVIFAPAVVPLITRLEEQFTQYDIEQISGLSSAYAVRLYELLICWRTTGKTPVLDLTEFRKRLGVLDTEYTRTDNLKMRVIEQSLKQINKHTDITASYEQHKKGRTITGFSFKFKQKKKTEPETPKNNDSGVSKPKTVEIPAEVVKQPKNTNLSDLEKRVRMITGAIAKNNLASRFQHGNESPLDMMKRIQSEITSDETADLWQNKLESMGVVF

SEQ ID NO: 13 - DNA, 999 bp, artificial sequence
  codon-optimized MSBI1
atgagcgacctgatcgtgaaagacaatgccctgatgaacgcctcctacaacctggcactggtcgaacagagactgattctgctggctatcatcgaggcaagggagaccggcaagggcatcaacgccaatgaccccctgacagtgcacgccagctcctacatcaaccagtttaatgtggagcgccacaccgcctatcaggccctgaaggacgcctgcaaggatctgtttgcccggcagttcagctaccaggagaagcgggagagaggcaggatcaacatcacaagcagatgggtgtcccagatcggctatatggacgataccgccacagtggagatcatctttgcaccagcagtggtgcctctgatcaccaggctggaggagcagttcacacagtacgacatcgagcagatctccggactgtctagcgcctacgccgtgcgcatgtatgagctgctgatctgttggcggtctaccggcaagacacctatcatcgagctggatgagttccgcaagcggatcggcgtgctggacaccgagtacaccagaacagataacctgaagatgagagtgatcgagctggccctgaagcagatcaatgagcacaccgatatcacagcctcttatgagcagcacaagaagggccgcgtgatcaccggcttcagctttaagttcaagcacaagaagcagaactctgacaagacaccaaagaatagcgattcctctccccggatcgtgaagcacagccagatccctaccaacatcgtgaagcagccagagaatgccaagatgtccgacctggagcacagggcatctagggtgacaggcgagatcatgagaaataggctgagcgatcggttcaagcagggcgacgagtccgccatcgatatgatgaagagaatccagtccgagatcatcaccgacgccatcgccgatcagtgggaatctaaactggaagagtttggagtcgtgtttggagcacatcaccatcatcatcactga

SEQ ID NO: 14 - protein, 326 aa, artificial sequence
  MSBI1 protein
MSDLIVKDNALMNASYNLALVEQRLILLAIIEARETGKGINANDPLTVHASSYINQFNVERHTAYQALKDACKDLFARQFSYQEKRERGRINITSRWVSQIGYMDDTATVEIIFAPAVVPLITRLEEQFTQYDIEQISGLSSAYAVRMYELLICWRSTGKTPIIELDEFRKRIGVLDTEYTRTDNLKMRVIELALKQINEHTDITASYEQHKKGRVITGFSFKFKHKKQNSDKTPKNSDSSPRIVKHSQIPTNIVKQPENAKMSDLEHRASRVTGEIMRNRLSDRFKQGDESAIDMMKRIQSEIITDAIADQWESKLEEFGVVFGA

SEQ ID NO: 15 - DNA, 974 bp, artificial sequence
  MSBI1 wild type
atgagcgatttaatagtaaaagataacgccctaatgaatgctagttataacttagctttggttgaacagaggttaattctattagcaatcatagaagcgagagaaacaggcaaagggattaatgccaatgatcctttaacagttcatgcaagtagctatatcaatcaatttaacgtagaaaggcatacggcatatcaagccctcaaagatgcttgtaaagacttgtttgcccgtcaattcagttaccaagaaaagcgagaacgaggacgaattaatattacaagtcgatgggtttcgcaaattggctatatggacgatacagcaaccgttgagattatttttgcccctgcggttgttcctctgattacacggctagaggaacagttcacccagtacgatattgagcaaattagcggtttatcgagtgcatatgctgttcgtatgtacgaactgctgatttgttggcgtagcacaggcaaaacaccaattattgagctagacgagtttagaaagcgaataggtgttttagatactgaatacactagaacagataatttaaagatgcgagttattgaattagccctaaaacaaatcaacgaacatacagacatcacagcaagctatgaacaacacaaaaaagggcgagtgattacaggattctcattcaagtttaagcacaagaaacaaaacagcgataaaacgccaaaaaatagcgattctagcccacgtatcgtaaaacatagtcaaatccctccaacattgtaaaacagcctgaaaacgccaaaatgagcgatttagaacatagagcgagccgtgttacaggggaaataatgcgaaatcgtctgtcagatcggtttaaacaaggcgatgaatcagcaatcgacatgatgaaacgtattcaaagtgaaataataaccgatgcaatagcagaccagtgggaaagcaaactggaggagtttggcgtggttttttag